European Patent Application EP 4 789 682 A2, published August 12, 2026. Title: Antibody formulation. Applicant: Novartis AG. Application EP. The sequence listing filed with the application follows.

SEQUENCE LISTING (4 sequences)

SEQ ID NO: 1 - protein, 137 aa, Homo sapiens
MEFGLSWVFLVALLRGVQCQVQLVESGGGVVQPGRSLRLSCAASGFTFSVYGMNWVRQAPGKGLEWVAIIWYDGDNQYYADSVKGRFTISRDNSKNTLYLQMNGLRAEDTAVYYCARDLRTGPFDYWGQGTLVTVSS

SEQ ID NO: 2 - protein, 126 aa, Homo sapiens
MLPSQLIGFLLLWVPASRGEIVLTQSPDFQSVTPKEKVTITCRASQSIGSSLHWYQQKPDQSPKLLIKYASQSFSGVPSRFSGSGSGTDFTLTINSLEAEDAAAYYCHQSSSLPFTFGPGTKVDIK

SEQ ID NO: 3 - DNA, 410 bp, Homo sapiens
  source 1..410: mol_type = other DNA
atggagtttgggctgagctgggttttcctcgttgctcttttaagaggtgtccagtgtcaggtgcagctggtggagtctgggggaggcgtggtccagcctgggaggtccctgagactctcctgtgcagcgtctggattcaccttcagtgtttatggcatgaactgggtccgccaggctccaggcaaggggctggagtgggtggcaattatttggtatgatggagataatcaatactatgcagactccgtgaagggccgattcaccatctccagagacaattccaagaacacgctgtatctgcaaatgaacggcctgagagccgaggacacggctgtgtattattgtgcgagagatcttaggactgggccttttgactactggggccagggaaccctggtcaccgtctcctc

SEQ ID NO: 4 - DNA, 378 bp, Homo sapiens
  source 1..378: mol_type = other DNA
atgttgccatcacaactcattgggtttctgctgctctgggttccagcctccaggggtgaaattgtgctgactcagtctccagactttcagtctgtgactccaaaggagaaagtcaccatcacctgccgggccagtcagagcattggtagtagcttacactggtaccagcagaaaccagatcagtctccaaagctcctcatcaagtatgcttcccagtccttctcaggggtcccctcgaggttcagtggcagtggatctgggacagatttcaccctcaccatcaatagcctggaagctgaagatgctgcagcgtattactgtcatcagagtagtagtttaccattcactttcggccctgggaccaaagtggatatcaaa